European Patent Specification EP 3 684 813 B1, published October 8, 2025. Title: Agonistic CD40 antibodies. Applicant: Mab Discovery GmbH. The sequence listing filed with the application follows.

SEQUENCE LISTING (112 sequences)

SEQ ID NO: 1 - protein, 122 aa, Artificial Sequence
  humanized antibody sequence
EVQLEESGGDLVQPGASLRLSCAASGFSFSFSYWICWVRQAPGKGLELVSCIYTTSGSTYYASWAKGRFTISIDNSKTTLYLQMNSLRAEDTATYFCARSSGVSYPSYFHLWGQGTLVTVSS

SEQ ID NO: 2 - protein, 125 aa, Artificial Sequence
  humanized antibody sequence
EVQLEESGGGLVQPGASLRLSCAASGFSFSGYWMCWVRQAPGKGLEWVGCIYTNSGVTYYANWAKGRFTISKDTSKTTLYLQMNSLRAEDTATYFCARGGAIYNDYDYAFYYSLWGQGTLVTVSS

SEQ ID NO: 3 - protein, 117 aa, Artificial Sequence
  humanized antibody sequence
EVQLEESGGDLVQPGASLRLSCAASGFDFNSNAMSWVRQAPGKGLEWVASIYAGGSGSTYYASWAKGRFTISKDTSKTTLYLQMNSLRAEDTATYFCARGITRLPLWGQGTLVTVSS

SEQ ID NO: 4 - protein, 117 aa, Artificial Sequence
  humanized antibody sequence
EVQLEESGGDLVQPGASLRLSCAVSGFDFSSNAMSWVRQAPGKGLEWVSSIYAGSSGSTYYASWAKGRFTISKDASKTTLYLQMNSLRAEDTATYFCARGVTRLPLWGQGTLVTVSS

SEQ ID NO: 5 - protein, 117 aa, Artificial Sequence
  humanized antibody sequence
EVQLEESGGGLVQPGGSLRLSCAASGFDFSSNTMCWVRQAPGKGLEWVACIYAGSSGSTYYASWAKGRFTISKDISKTTLYLQMNSLRAEDTATYFCARGLSRFSLWGQGTLVTVSS

SEQ ID NO: 6 - protein, 117 aa, Artificial Sequence
  humanized antibody sequence
EVQLEESGGGLVQPGGSLRLSCAASGFDFSTNAVSWVRQAPGKGLEWVGSISAGSSGSTYYASWAKGRFTISKDTSKTTLYLQMNSLRAEDTATYFCARGYTYLTLWGQGTLVTVSS

SEQ ID NO: 7 - protein, 117 aa, Artificial Sequence
  humanized antibody sequence
EVQLEESGGGLVQPGGSLRLSCAASGFSFSSNAMSWVRQAPGKGPEWVVTIYAGSSGSTYYASWAKGRFTISKDTSKTTLYLQMNSLRAEDTATYFCARGATYLTLWGQGTLVTVSS

SEQ ID NO: 8 - protein, 117 aa, Artificial Sequence
  humanized antibody sequence
EVQLVESGGGLVQPGGSLRLSCAASGFDFSSNAMSWVRQAPGKGLEWVGIIYAGSSGSTYYASWAKGRFTISKDTSKTTLYLQMNSLRAEDTATYFCARGATYITLWGQGTLVTVSS

SEQ ID NO: 9 - protein, 117 aa, Artificial Sequence
  humanized antibody sequence
EVQLEESGGGLVQPGGSLRLSCAASGFDFSSNAMSWVRQAPGKGLEWVGTIYAGSNGNTDYASWAKGRFTISKDTSKTTLYLQMNSLRAEDTATYFCARGASYFTLWGQGTLVTVSS

SEQ ID NO: 10 - protein, 117 aa, Artificial Sequence
  humanized antibody sequence
EVQLEESGGGLVQPGGSLRLSCAASGFDFSTNAMCWVRQAPGKGLEWVACIAAGSSIITYYASWAKGRFTISKDTSKTTLYLQMNSLRAEDTAVYFCARGLSRFALWGQGTLVTVSS

SEQ ID NO: 11 - protein, 123 aa, Artificial Sequence
  humanized antibody sequence
EVQLEESGGGLVQPGGSLRLSCAASGIDFSRYYYMCWVRQAPGKGPEWVACYSNGDGSTYYASWAKGRFTISKDTSKTTLYLQMNSLRAEDTATYFCARGADYSAGAAAFNLWGQGTLVTVSS

SEQ ID NO: 12 - protein, 123 aa, Artificial Sequence
  humanized antibody sequence
EVQLEESGGGLVQPGGSLRLSCAASGIDFSRYYYICWVRQAPGKGPEWVACFANGDGSTYYASWAKGRFTISKDTSKTTLYLQMNSLRAEDTATYFCARGADYSGGAAAFNLWGQGTLVTVSS

SEQ ID NO: 13 - protein, 126 aa, Artificial Sequence
  humanized antibody sequence
EVQLEESGGGLVQPGGSLRLSCAASGIDFSRYFYMCWVRQAPGKGLEWVACIGPGVSGDTYYASWAKGRFTISGDTSKTTLYLQMNSLRAEDTATYFCARGVDYTYGDAGAAFNLWGQGTLVTVSS

SEQ ID NO: 14 - protein, 125 aa, Artificial Sequence
  humanized antibody sequence
EVQLEESGGGLVQPGASLRLSCAASGIDFSRYFYVCWVRQAPGKGLEWVGCFANHDDSIYYAGWMNGRFTISKDTSKTTLYLQMNSLRAEDTATYFCARGVDYTVGYGGAAFNLWGQGTLVTVSS

SEQ ID NO: 15 - protein, 112 aa, Artificial Sequence
  humanized antibody sequence
DIQMTQSPSSLSASVGDRVTITCQASQSISSYLAWYQQKPGQAPKLLIYSASKLPSGVPSRFSGSGSGTDFTLTISSLQPEDFATYHCQTYYYSSSSSYDYGFGQGTKVVIK

SEQ ID NO: 16 - protein, 111 aa, Artificial Sequence
  humanized antibody sequence
DIVMTQSPSSLSASVGDRVTITCQASQSISSYLAWYQQKPGQAPKLLIYKASTLASGVPSRFSGSGSGTDFTLTISSLQPEDFATYYCQSYYGSSSISYNAFGQGTKVVIK

SEQ ID NO: 17 - protein, 110 aa, Artificial Sequence
  humanized antibody sequence
DIQMTQSPSSLSASVGDRVTITCQASQSISSYLAWYQQKPGQAPKLLIYDASKLASGVPSRFSGSGSGTDFTLTISSLQPEDFATYYCQGTYYGSTTISAFGQGTKVVIK

SEQ ID NO: 18 - protein, 110 aa, Artificial Sequence
  humanized antibody sequence
DIVMTQSPSSLSASVGDRVTITCQASQSISSYLAWYQQKPGQAPKLLIYDASTLASGVPSRFSGSGSGTDFTLTISSLQPEDFATYYCQGTVYGSSTISAFGQGTKVVIK

SEQ ID NO: 19 - protein, 111 aa, Artificial Sequence
  humanized antibody sequence
DIVMTQSPSSLSASVGDRVTITCQASQSISNYLAWYQQKPGQAPKLLIYDASKLASGVPSRFSGSGSGTDFTLTISSLQPEDFATYYCQGGDYYGSSYVVAFGGGTKVVIK

SEQ ID NO: 20 - protein, 111 aa, Artificial Sequence
  humanized antibody sequence
DIVMTQSPSSLSASVGDRVTITCQASHSISSTYLSWYQQKPGQAPKLLIYRASTLASGVPSRFSGSGSGTDFTLTISSLQPEDFATYYCQYTDYGSSYVSTFGQGTKVVIK

SEQ ID NO: 21 - protein, 112 aa, Artificial Sequence
  humanized antibody sequence
DIVMTQSPSSLSASVGDRVTITCQASQSISNYLSWYQQKPGQAPKLLIYRASTLPSGVPSRFSGSGSGTDFTLTISSLQPEDFATYYCQGYYYSGTTYDSTAFGQGTKVVIK

SEQ ID NO: 22 - protein, 114 aa, Artificial Sequence
  humanized antibody sequence
DIVMTQSPSSLSASVGDRVTITCQASQSIGSYLAWYQQKPGQAPKLLIYRASTLASGVPSRFSGSGSGTDFTLTISSLQPEDFATYYCQGYYYSTTTTTYDSSAFGQGTKVVIK

SEQ ID NO: 23 - protein, 112 aa, Artificial Sequence
  humanized antibody sequence
DIVMTQSPSSLSASVGDRVTITCQASESVVSNNRLAWYQQKPGQAPKLLIYLASTLPSGVPSRFSGSGSGTDFTLTISSLQPEDFATYYCAGYKSSSTDGTAFGQGTKVVIK

SEQ ID NO: 24 - protein, 111 aa, Artificial Sequence
  humanized antibody sequence
DIVMTQSPSSLSASVGDRVTITCQASQSISSYLSWYQQKPGQAPKLLIYLTSTLASGVPSRFSGSGSGTDFTLTISSLQPEDFATYYCQGYYSSSSYVSNGFGQGTKVVIK

SEQ ID NO: 25 - protein, 110 aa, Artificial Sequence
  humanized antibody sequence
DIQMTQSPSSLSASVGDRVTITCQASESIGNALVWYQQKPGQAPKLLIYRASILASGVPSRFSGSGSGTDFTLTISSLQPEDFATYYCQDYYGSSTEYNTFGQGTKVVIK

SEQ ID NO: 26 - protein, 110 aa, Artificial Sequence
  humanized antibody sequence
DIQMTQSPSSLSASVGDRVTITCQASQSISSRLAWYQQKPGQAPKLLIYRASTLASGVPSRFSGSGSGTDFTLTISSLQPEDFATYYCQDYYGSSTEYNAFGQGTKVVIK

SEQ ID NO: 27 - protein, 114 aa, Artificial Sequence
  humanized antibody sequence
DIVMTQSPSSLSASVGDRVTITCQASQSISSYLAWYQQKPGQAPKLLIYRASILASGVPSRFSGSGSGTDFTLTISSLQPEDFATYYCQTYYSSRTYSYGSPNAFGQGTKVVIK

SEQ ID NO: 28 - protein, 109 aa, Artificial Sequence
  humanized antibody sequence
DIVMTQSPSSLSASVGDRVTITCQASQSIGSYLSWYQQKPGQAPKLLIYRATTLASGVPSRFSGSGSGTDFTLTISSLQPEDFATYYCQSYYRDSSSSAFGQGTKVVIK

SEQ ID NO: 29 - protein, 6 aa, Artificial Sequence
  CDR
FSYWIC

SEQ ID NO: 30 - protein, 5 aa, Artificial Sequence
  CDR
GYWMC

SEQ ID NO: 31 - protein, 5 aa, Artificial Sequence
  humanized antibody sequence
SNAMS

SEQ ID NO: 32 - protein, 5 aa, Artificial Sequence
  humanized antibody sequence
SNAMS

SEQ ID NO: 33 - protein, 5 aa, Artificial Sequence
  humanized antibody sequences
SNTMC

SEQ ID NO: 34 - protein, 5 aa, Artificial Sequence
  humanized antibody sequence
TNAVS

SEQ ID NO: 35 - protein, 5 aa, Artificial Sequence
  humanized antibody sequence
SNAMS

SEQ ID NO: 36 - protein, 5 aa, Artificial Sequence
  humanized antibody sequence
SNAMS

SEQ ID NO: 37 - protein, 5 aa, Artificial Sequence
  humanized antibody sequence
SNAMS

SEQ ID NO: 38 - protein, 5 aa, Artificial Sequence
  humanized antibody sequence
TNAMC

SEQ ID NO: 39 - protein, 6 aa, Artificial Sequence
  humanized antibody sequence
RYYYMC

SEQ ID NO: 40 - protein, 6 aa, Artificial Sequence
  humanized antibody sequence
RYYYIC

SEQ ID NO: 41 - protein, 6 aa, Artificial Sequence
  humanized antibody sequence
RYFYMC

SEQ ID NO: 42 - protein, 6 aa, Artificial Sequence
  humanized antibody sequence
RYFYVC

SEQ ID NO: 43 - protein, 17 aa, Artificial Sequence
  humanized antibody sequence
CIYTTSGSTYYASWAKG

SEQ ID NO: 44 - protein, 17 aa, Artificial Sequence
  humanized antibody sequence
CIYTNSGVTYYANWAKG

SEQ ID NO: 45 - protein, 18 aa, Artificial Sequence
  humanized antibody sequence
SIYAGGSGSTYYASWAKG

SEQ ID NO: 46 - protein, 18 aa, Artificial Sequence
  humanized antibody sequence
SIYAGSSGSTYYASWAKG

SEQ ID NO: 47 - protein, 18 aa, Artificial Sequence
  humanized antibody sequence
CIYAGSSGSTYYASWAKG

SEQ ID NO: 48 - protein, 18 aa, Artificial Sequence
  humanized antibody sequence
SISAGSSGSTYYASWAKG

SEQ ID NO: 49 - protein, 18 aa, Artificial Sequence
  humanized antibody sequence
TIYAGSSGSTYYASWAKG

SEQ ID NO: 50 - protein, 18 aa, Artificial Sequence
  humanized antibody sequence
IIYAGSSGSTYYASWAKG

SEQ ID NO: 51 - protein, 18 aa, Artificial Sequence
  humanized antibody sequence
TIYAGSNGNTDYASWAKG

SEQ ID NO: 52 - protein, 18 aa, Artificial Sequence
  humanized antibody sequence
CIAAGSSIITYYASWAKG

SEQ ID NO: 53 - protein, 17 aa, Artificial Sequence
  humanized antibody sequence
CYSNGDGSTYYASWAKG

SEQ ID NO: 54 - protein, 17 aa, Artificial Sequence
  humanized antibody sequence
CFANGDGSTYYASWAKG

SEQ ID NO: 55 - protein, 18 aa, Artificial Sequence
  humanized antibody sequence
CIGPGVSGDTYYASWAKG

SEQ ID NO: 56 - protein, 17 aa, Artificial Sequence
  humanized antibody sequence
CFANHDDSIYYAGWMNG

SEQ ID NO: 57 - protein, 12 aa, Artificial Sequence
  humanized antibody sequence
SSGVSYPSYFHL

SEQ ID NO: 58 - protein, 16 aa, Artificial Sequence
  humanized antibody sequence
GGAIYNDYDYAFYYSL

SEQ ID NO: 59 - protein, 7 aa, Artificial Sequence
  humanized antibody sequence
GITRLPL

SEQ ID NO: 60 - protein, 7 aa, Artificial Sequence
  humanized antibody sequence
GVTRLPL

SEQ ID NO: 61 - protein, 7 aa, Artificial Sequence
  humanized antibody sequence
GLSRFSL

SEQ ID NO: 62 - protein, 7 aa, Artificial Sequence
  humanized antibody sequence
GYTYLTL

SEQ ID NO: 63 - protein, 7 aa, Artificial Sequence
  humanized antibody sequence
GATYLTL

SEQ ID NO: 64 - protein, 7 aa, Artificial Sequence
  humanized antibody sequence
GATYITL

SEQ ID NO: 65 - protein, 7 aa, Artificial Sequence
  humanized antibody sequence
GASYFTL

SEQ ID NO: 66 - protein, 7 aa, Artificial Sequence
  humanized antibody sequence
GLSRFAL

SEQ ID NO: 67 - protein, 13 aa, Artificial Sequence
  humanized antibody sequence
GADYSAGAAAFNL

SEQ ID NO: 68 - protein, 13 aa, Artificial Sequence
  humanized antibody sequence
GADYSGGAAAFNL

SEQ ID NO: 69 - protein, 15 aa, Artificial Sequence
  humanized antibody sequence
GVDYTYGDAGAAFNL

SEQ ID NO: 70 - protein, 15 aa, Artificial Sequence
  humanized antibody sequence
GVDYTVGYGGAAFNL

SEQ ID NO: 71 - protein, 11 aa, Artificial Sequence
  humanized antibody sequence
QASQSISSYLA

SEQ ID NO: 72 - protein, 11 aa, Artificial Sequence
  humanized antibody sequence
QASQSISSYLA

SEQ ID NO: 73 - protein, 11 aa, Artificial Sequence
  humanized antibody sequence
QASQSISSYLA

SEQ ID NO: 74 - protein, 11 aa, Artificial Sequence
  humanized antibody sequence
QASQSISSYLA

SEQ ID NO: 75 - protein, 11 aa, Artificial Sequence
  humanized antibody sequence
QASQSISNYLA

SEQ ID NO: 76 - protein, 12 aa, Artificial Sequence
  humanized antibody sequence
QASHSISSTYLS

SEQ ID NO: 77 - protein, 11 aa, Artificial Sequence
  humanized antibody sequence
QASQSISNYLS

SEQ ID NO: 78 - protein, 11 aa, Artificial Sequence
  humanized antibody sequence
QASQSIGSYLA

SEQ ID NO: 79 - protein, 13 aa, Artificial Sequence
  humanized antibody sequence
QASESVVSNNRLA

SEQ ID NO: 80 - protein, 11 aa, Artificial Sequence
  humanized antibody sequence
QASQSISSYLS

SEQ ID NO: 81 - protein, 11 aa, Artificial Sequence
  humanized antibody sequence
QASESIGNALV

SEQ ID NO: 82 - protein, 11 aa, Artificial Sequence
  humanized antibody sequence
QASQSISSRLA

SEQ ID NO: 83 - protein, 11 aa, Artificial Sequence
  humanized antibody sequence
QASQSISSYLA

SEQ ID NO: 84 - protein, 11 aa, Artificial Sequence
  humanized antibody sequence
QASQSIGSYLS

SEQ ID NO: 85 - protein, 7 aa, Artificial Sequence
  humanized antibody sequence
SASKLPS

SEQ ID NO: 86 - protein, 7 aa, Artificial Sequence
  humanized antibody sequence
KASTLAS

SEQ ID NO: 87 - protein, 7 aa, Artificial Sequence
  humanized antibody sequence
DASKLAS

SEQ ID NO: 88 - protein, 7 aa, Artificial Sequence
  humanized antibody sequence
DASTLAS

SEQ ID NO: 89 - protein, 7 aa, Artificial Sequence
  humanized antibody sequence
DASKLAS

SEQ ID NO: 90 - protein, 7 aa, Artificial Sequence
  humanized antibody sequence
RASTLAS

SEQ ID NO: 91 - protein, 7 aa, Artificial Sequence
  humanized antibody sequence
RASTLPS

SEQ ID NO: 92 - protein, 7 aa, Artificial Sequence
  humanized antibody sequence
RASTLAS

SEQ ID NO: 93 - protein, 7 aa, Artificial Sequence
  humanized antibody sequence
LASTLPS

SEQ ID NO: 94 - protein, 7 aa, Artificial Sequence
  humanized antibody sequence
LTSTLAS

SEQ ID NO: 95 - protein, 7 aa, Artificial Sequence
  humanized antibody sequence
RASILAS

SEQ ID NO: 96 - protein, 7 aa, Artificial Sequence
  humanized antibody sequence
RASTLAS

SEQ ID NO: 97 - protein, 7 aa, Artificial Sequence
  humanized antibody sequence
RASILAS

SEQ ID NO: 98 - protein, 7 aa, Artificial Sequence
  humanized antibody sequence
RATTLAS

SEQ ID NO: 99 - protein, 14 aa, Artificial Sequence
  humanized antibody sequence
QTYYYSSSSSYDYG

SEQ ID NO: 100 - protein, 13 aa, Artificial Sequence
  humanized antibody sequence
QSYYGSSSISYNA

SEQ ID NO: 101 - protein, 12 aa, Artificial Sequence
  humanized antibody sequence
QGTYYGSTTISA

SEQ ID NO: 102 - protein, 12 aa, Artificial Sequence
  humanized antibody sequence
QGTVYGSSTISA

SEQ ID NO: 103 - protein, 13 aa, Artificial Sequence
  humanized antibody sequence
QGGDYYGSSYVVA

SEQ ID NO: 104 - protein, 12 aa, Artificial Sequence
  humanized antibody sequence
QYTDYGSSYVST

SEQ ID NO: 105 - protein, 14 aa, Artificial Sequence
  humanized antibody sequence
QGYYYSGTTYDSTA

SEQ ID NO: 106 - protein, 16 aa, Artificial Sequence
  humanized antibody sequence
QGYYYSTTTTTYDSSA

SEQ ID NO: 107 - protein, 12 aa, Artificial Sequence
  humanized antibody sequence
AGYKSSSTDGTA

SEQ ID NO: 108 - protein, 13 aa, Artificial Sequence
  humanized antibody sequence
QGYYSSSSYVSNG

SEQ ID NO: 109 - protein, 12 aa, Artificial Sequence
  humanized antibody sequence
QDYYGSSTEYNT

SEQ ID NO: 110 - protein, 12 aa, Artificial Sequence
  humanized antibody sequence
QDYYGSSTEYNA

SEQ ID NO: 111 - protein, 16 aa, Artificial Sequence
  humanized antibody sequence
QTYYSSRTYSYGSPNA

SEQ ID NO: 112 - protein, 11 aa, Artificial Sequence
  CDR
QSYYRDSSSSA